European Patent Application EP 4 775 219 A1, published July 15, 2026. Title: 病毒3C蛋白酶用于预防或治疗肿瘤的用途. Applicant: 中国人民解放军军事科学院军事医学研究院. The sequence listing filed with the application follows.

SEQUENCE LISTING (7 sequences)

SEQ ID NO: 1 - protein, 183 aa, unidentified
GPSLDFALSLLRRNIRQVQTDQGHFTMLGVRDRLAVLPRHSQPGKTIWIEHKLVNVLDAVELVDEQGVNLELTLITLDTNEKFRDITKFIPENISTASDATLVINTEHMPSMFVPVGDVVQYGFLNLSGKPTHRTMMYNFPTKAGQCGGVVTSVGKVIGIHIGGNGRQGFCAGLKRSYFASEQ

SEQ ID NO: 2 - RNA, 1017 nt, synthetic construct
  source 1..1017: mol_type = other RNA
gggaataaactagtattcttctggtccccacagactcagagagaacccgccaccatgggccccagcctggacttcgccctgagcctgctgcggagaaatatccggcaggtgcagaccgatcaaggccactttacaatgctgggcgtgagagaccggctcgccgtgctgcctcgccactcccagcctggaaagaccatttggatcgagcataagctggtgaacgtgctggatgccgtggaactggtcgacgagcagggcgtgaacctggagctgacactgatcaccctggacaccaacgagaagttccgggacatcaccaaattcatccccgaaaacatcagcaccgcctccgatgctacactggtgatcaacaccgagcacatgcctagcatgttcgtgcccgtgggcgacgtggtgcagtacggcttcctgaacctgagcggcaagccaacccaccggacaatgatgtacaatttccctacaaaggccggacagtgcggcggggtggtgacctctgtgggcaaggtgatcggcatccacatcggcggcaacggaaggcagggcttttgtgccggcctgaagagaagctacttcgccagcgagcagtgatgactcgagctggtactgcatgcacgcaatgctagctgcccctttcccgtcctgggtaccccgagtctcccccgacctcgggtcccaggtatgctcccacctccacctgccccactcaccacctctgctagttccagacacctcccaagcacgcagcaatgcagctcaaaacgcttagcctagccacacccccacgggaaacagcagtgattaacctttagcaataaacgaaagtttaactaagctatactaaccccagggttggtcaatttcgtgccagccacaccctggagctagcaaaaaaaaaaaaaaaaaaaaaaaaaaaaaagcatatgactaaaaaaaaaaaaaaaaaaaaaaaaaaaaaaaaaaaaaaaaaaaaaaaaaaaaaaaaaaaaaaaaaaaaaa

SEQ ID NO: 3 - RNA, 549 nt, synthetic construct
  source 1..549: mol_type = other RNA
ggccccagcctggacttcgccctgagcctgctgcggagaaatatccggcaggtgcagaccgatcaaggccactttacaatgctgggcgtgagagaccggctcgccgtgctgcctcgccactcccagcctggaaagaccatttggatcgagcataagctggtgaacgtgctggatgccgtggaactggtcgacgagcagggcgtgaacctggagctgacactgatcaccctggacaccaacgagaagttccgggacatcaccaaattcatccccgaaaacatcagcaccgcctccgatgctacactggtgatcaacaccgagcacatgcctagcatgttcgtgcccgtgggcgacgtggtgcagtacggcttcctgaacctgagcggcaagccaacccaccggacaatgatgtacaatttccctacaaaggccggacagtgcggcggggtggtgacctctgtgggcaaggtgatcggcatccacatcggcggcaacggaaggcagggcttttgtgccggcctgaagagaagctacttcgccagcgagcag

SEQ ID NO: 4 - RNA, 48 nt, synthetic construct
  source 1..48: mol_type = other RNA
gggaataaactagtattcttctggtccccacagactcagagagaaccc

SEQ ID NO: 5 - skipped

SEQ ID NO: 6 - RNA, 295 nt, synthetic construct
  source 1..295: mol_type = other RNA
ctcgagctggtactgcatgcacgcaatgctagctgcccctttcccgtcctgggtaccccgagtctcccccgacctcgggtcccaggtatgctcccacctccacctgccccactcaccacctctgctagttccagacacctcccaagcacgcagcaatgcagctcaaaacgcttagcctagccacacccccacgggaaacagcagtgattaacctttagcaataaacgaaagtttaactaagctatactaaccccagggttggtcaatttcgtgccagccacaccctggagctagc

SEQ ID NO: 7 - RNA, 110 nt, synthetic construct
  source 1..110: mol_type = other RNA
aaaaaaaaaaaaaaaaaaaaaaaaaaaaaagcatatgactaaaaaaaaaaaaaaaaaaaaaaaaaaaaaaaaaaaaaaaaaaaaaaaaaaaaaaaaaaaaaaaaaaaaaa